European Patent Specification EP 4 003 348 B1, published April 3, 2024. Title: Compounds And Methods For Treating Fibrotic Pathologies. Applicant: Mayo Foundation for Medical Education and Research. The sequence listing filed with the application follows.

SEQUENCE LISTING (54 sequences)

SEQ ID NO: 1 - DNA, 22 bp, Artificial
  synthetic oligonucleotide primer
cccagccctatcagtcatattg

SEQ ID NO: 2 - DNA, 21 bp, Artificial
  synthetic oligonucleotide primer
aggattcatctgcgagttcag

SEQ ID NO: 3 - DNA, 17 bp, Artificial
  synthetic oligonucleotide primer
gtccagcacgaggctca

SEQ ID NO: 4 - DNA, 17 bp, Artificial
  synthetic oligonucleotide primer
tcgccttcgtggtcctc

SEQ ID NO: 5 - DNA, 23 bp, Artificial
  synthetic oligonucleotide primer
aagggacacagaggtttcagtgg

SEQ ID NO: 6 - DNA, 24 bp, Artificial
  synthetic oligonucleotide primer
cagcaccagtagcaccatcatttc

SEQ ID NO: 7 - DNA, 21 bp, Artificial
  synthetic oligonucleotide primer
gtgaagaagaggacagcactg

SEQ ID NO: 8 - DNA, 18 bp, Artificial
  synthetic oligonucleotide primer
cccattcccaccatcacc

SEQ ID NO: 9 - DNA, 20 bp, Artificial
  synthetic oligonucleotide primer
tgtcagtcaaagcaagcccg

SEQ ID NO: 10 - DNA, 24 bp, Artificial
  synthetic oligonucleotide primer
ttaggacgctcataagtgtcaccc

SEQ ID NO: 11 - DNA, 21 bp, Artificial
  synthetic oligonucleotide primer
tcagctacaatgggatcttgg

SEQ ID NO: 12 - DNA, 21 bp, Artificial
  synthetic oligonucleotide primer
tcagctacaatgggatcttgg

SEQ ID NO: 13 - DNA, 21 bp, Artificial
  synthetic oligonucleotide primer
acattcgctacacaggacatc

SEQ ID NO: 14 - DNA, 20 bp, Artificial
  synthetic oligonucleotide primer
ttcccacttcagaacaccag

SEQ ID NO: 15 - DNA, 20 bp, Artificial
  synthetic oligonucleotide primer
tgccagtggatcgacataac

SEQ ID NO: 16 - DNA, 21 bp, Artificial
  synthetic oligonucleotide primer
gaaacgtagcgacctgtgtag

SEQ ID NO: 17 - DNA, 20 bp, Artificial
  synthetic oligonucleotide primer
gtgcagcgacaaaaggattc

SEQ ID NO: 18 - DNA, 19 bp, Artificial
  synthetic oligonucleotide primer
gcggtaggttgagaggatg

SEQ ID NO: 19 - DNA, 19 bp, Artificial
  synthetic oligonucleotide primer
agcgaaaagagggtcaacg

SEQ ID NO: 20 - DNA, 22 bp, Artificial
  synthetic oligonucleotide primer
tgtcattggcacgatagaactc

SEQ ID NO: 21 - DNA, 21 bp, Artificial
  synthetic oligonucleotide primer
gtggcagagtcagatttctcc

SEQ ID NO: 22 - DNA, 20 bp, Artificial
  synthetic oligonucleotide primer
ttgttcctgagacgctgttc

SEQ ID NO: 23 - DNA, 21 bp, Artificial
  synthetic oligonucleotide primer
gggagatgaagtttgaggtgg

SEQ ID NO: 24 - DNA, 21 bp, Artificial
  synthetic oligonucleotide primer
agatggtctgtatagtccggg

SEQ ID NO: 25 - DNA, 22 bp, Artificial
  synthetic oligonucleotide primer
aaacccagatcgagactcaaag

SEQ ID NO: 26 - DNA, 20 bp, Artificial
  synthetic oligonucleotide primer
acccattcccaaagtagcag

SEQ ID NO: 27 - DNA, 23 bp, Artificial
  synthetic oligonucleotide primer
ctccttccagttttacagcaaag

SEQ ID NO: 28 - DNA, 19 bp, Artificial
  synthetic oligonucleotide primer
tttccccagttttctcccc

SEQ ID NO: 29 - DNA, 21 bp, Artificial
  synthetic oligonucleotide primer
tgcctaccgacaagattgatg

SEQ ID NO: 30 - DNA, 21 bp, Artificial
  synthetic oligonucleotide primer
atcccttcccagactttgatg

SEQ ID NO: 31 - DNA, 21 bp, Artificial
  synthetic oligonucleotide primer
cccgtagccattatgatcgtc

SEQ ID NO: 32 - DNA, 20 bp, Artificial
  synthetic oligonucleotide primer
agagcattcgacagggtttc

SEQ ID NO: 33 - DNA, 21 bp, Artificial
  synthetic oligonucleotide primer
tccttctaccacctcagcgag

SEQ ID NO: 34 - DNA, 23 bp, Artificial
  synthetic oligonucleotide primer
ccggatggtcactctttaggaag

SEQ ID NO: 35 - DNA, 20 bp, Artificial
  synthetic oligonucleotide primer
ttgctccaaactggcgtcta

SEQ ID NO: 36 - DNA, 21 bp, Artificial
  synthetic oligonucleotide primer
acgtgatctccgtgtccttgt

SEQ ID NO: 37 - DNA, 21 bp, Artificial
  synthetic oligonucleotide primer
ctgccagtccgaaaatggaac

SEQ ID NO: 38 - DNA, 20 bp, Artificial
  synthetic oligonucleotide primer
cttcatccactggggctatc

SEQ ID NO: 39 - DNA, 23 bp, Artificial
  synthetic oligonucleotide primer
gacagagttagtgaatggagacc

SEQ ID NO: 40 - DNA, 21 bp, Artificial
  synthetic oligonucleotide primer
aaaagttcggagagtgtaggc

SEQ ID NO: 41 - DNA, 18 bp, Artificial
  synthetic oligonucleotide primer
gagaagcccagccagtcg

SEQ ID NO: 42 - DNA, 18 bp, Artificial
  synthetic oligonucleotide primer
ctcttgctctgggcttca

SEQ ID NO: 43 - DNA, 17 bp, Artificial
  synthetic oligonucleotide primer
cctgcgacccacacaag

SEQ ID NO: 44 - DNA, 18 bp, Artificial
  synthetic oligonucleotide primer
gacccaccgaagacacag

SEQ ID NO: 45 - DNA, 21 bp, Artificial
  synthetic oligonucleotide primer
ccagcagcatgatcaaaacac

SEQ ID NO: 46 - DNA, 22 bp, Artificial
  synthetic oligonucleotide primer
ggtggctacatgttagagtgtc

SEQ ID NO: 47 - DNA, 22 bp, Artificial
  synthetic oligonucleotide primer
atcatagccataggacatctgg

SEQ ID NO: 48 - DNA, 18 bp, Artificial
  synthetic oligonucleotide primer
ctggacagcctggacttc

SEQ ID NO: 49 - DNA, 21 bp, Artificial
  synthetic oligonucleotide primer
ctctgagtgatcctctggttc

SEQ ID NO: 50 - DNA, 23 bp, Artificial
  synthetic oligonucleotide primer
ccataagaacaagaccacatcct

SEQ ID NO: 51 - DNA, 20 bp, Artificial
  synthetic oligonucleotide primer
cttgctggtgttggtgattc

SEQ ID NO: 52 - DNA, 22 bp, Artificial
  synthetic oligonucleotide primer
atcagcctctgaatcatgtgaa

SEQ ID NO: 53 - DNA, 21 bp, Artificial
  synthetic oligonucleotide primer
tgctttttccaggggtgtgtt

SEQ ID NO: 54 - DNA, 23 bp, Artificial
  synthetic oligonucleotide primer
ttacttcctgcactaatttggca